European Patent Application EP 4 450 073 A1, published October 23, 2024. Title: Suppressor of intestinal tumor, suppressor of PGE2 production, and accelerator of IL-22BP production. Applicant: TOKYO UNIVERSITY OF SCIENCE FOUNDATION. The sequence listing filed with the application follows.

SEQUENCE LISTING (74 sequences)

SEQ ID NO: 1 - DNA, 22 bp, synthetic construct
  misc_feature 1..22: note = synthesized primer
  source 1..22: mol_type = other DNA
gacttcagcactcaagacatcc

SEQ ID NO: 2 - DNA, 21 bp, synthetic construct
  misc_feature 1..21: note = synthesized primer
  source 1..21: mol_type = other DNA
ttgtgtcgccaaaatgctagg

SEQ ID NO: 3 - DNA, 25 bp, synthetic construct
  misc_feature 1..25: note = synthesized primer
  source 1..25: mol_type = other DNA
caaccaacaagtgatattctccatg

SEQ ID NO: 4 - DNA, 21 bp, synthetic construct
  misc_feature 1..21: note = synthesized primer
  source 1..21: mol_type = other DNA
gatccacactctccagctgca

SEQ ID NO: 5 - DNA, 23 bp, synthetic construct
  misc_feature 1..23: note = synthesized primer
  source 1..23: mol_type = other DNA
gaggataccactcccaacagacc

SEQ ID NO: 6 - DNA, 24 bp, synthetic construct
  misc_feature 1..24: note = synthesized primer
  source 1..24: mol_type = other DNA
aagtgcatcatcgttgttcataca

SEQ ID NO: 7 - DNA, 23 bp, synthetic construct
  misc_feature 1..23: note = synthesized primer
  source 1..23: mol_type = other DNA
actgtacaaccgcagtaatacgc

SEQ ID NO: 8 - DNA, 23 bp, synthetic construct
  misc_feature 1..23: note = synthesized primer
  source 1..23: mol_type = other DNA
agtgaacattacagatttatccc

SEQ ID NO: 9 - DNA, 23 bp, synthetic construct
  misc_feature 1..23: note = synthesized primer
  source 1..23: mol_type = other DNA
cctacttcagcatcctctactgg

SEQ ID NO: 10 - DNA, 21 bp, synthetic construct
  misc_feature 1..21: note = synthesized primer
  source 1..21: mol_type = other DNA
agggtttcttgagaaggggac

SEQ ID NO: 11 - DNA, 22 bp, synthetic construct
  misc_feature 1..22: note = synthesized primer
  source 1..22: mol_type = other DNA
cattgccttctaggtctcctca

SEQ ID NO: 12 - DNA, 20 bp, synthetic construct
  misc_feature 1..20: note = synthesized primer
  source 1..20: mol_type = other DNA
cctgcttgccagtgcaaaat

SEQ ID NO: 13 - DNA, 21 bp, synthetic construct
  misc_feature 1..21: note = synthesized primer
  source 1..21: mol_type = other DNA
atgagtcgaaggagtctctcg

SEQ ID NO: 14 - DNA, 22 bp, synthetic construct
  misc_feature 1..22: note = synthesized primer
  source 1..22: mol_type = other DNA
gcacggatagtaacaacaggga

SEQ ID NO: 15 - DNA, 22 bp, synthetic construct
  misc_feature 1..22: note = synthesized primer
  source 1..22: mol_type = other DNA
ttcaacacactctatcactggc

SEQ ID NO: 16 - DNA, 21 bp, synthetic construct
  misc_feature 1..21: note = synthesized primer
  source 1..21: mol_type = other DNA
agaagcgtttgcggtactcat

SEQ ID NO: 17 - DNA, 19 bp, synthetic construct
  misc_feature 1..19: note = synthesized primer
  source 1..19: mol_type = other DNA
cctcgacttccactccctg

SEQ ID NO: 18 - DNA, 23 bp, synthetic construct
  misc_feature 1..23: note = synthesized primer
  source 1..23: mol_type = other DNA
tgagggcactaatgatgacagag

SEQ ID NO: 19 - DNA, 22 bp, synthetic construct
  misc_feature 1..22: note = synthesized primer
  source 1..22: mol_type = other DNA
tgtttgcgaaaaggagaatccg

SEQ ID NO: 20 - DNA, 23 bp, synthetic construct
  misc_feature 1..23: note = synthesized primer
  source 1..23: mol_type = other DNA
ccatgtgatccatcatctcagag

SEQ ID NO: 21 - DNA, 19 bp, synthetic construct
  misc_feature 1..19: note = synthesized primer
  source 1..19: mol_type = other DNA
gcaaagctgcggtgctatg

SEQ ID NO: 22 - DNA, 21 bp, synthetic construct
  misc_feature 1..21: note = synthesized primer
  source 1..21: mol_type = other DNA
tcacacaagtcaccccttctc

SEQ ID NO: 23 - DNA, 23 bp, synthetic construct
  misc_feature 1..23: note = synthesized primer
  source 1..23: mol_type = other DNA
atacttgtcggatttaggaggct

SEQ ID NO: 24 - DNA, 22 bp, synthetic construct
  misc_feature 1..22: note = synthesized primer
  source 1..22: mol_type = other DNA
gggcctatcttccaaatgaaca

SEQ ID NO: 25 - DNA, 20 bp, synthetic construct
  misc_feature 1..20: note = synthesized primer
  source 1..20: mol_type = other DNA
acttggaagttaggccctgc

SEQ ID NO: 26 - DNA, 22 bp, synthetic construct
  misc_feature 1..22: note = synthesized primer
  source 1..22: mol_type = other DNA
tgtgaaggacactttgtcgatg

SEQ ID NO: 27 - DNA, 21 bp, synthetic construct
  misc_feature 1..21: note = synthesized primer
  source 1..21: mol_type = other DNA
tgggtcgagtgtctttgtgtg

SEQ ID NO: 28 - DNA, 21 bp, synthetic construct
  misc_feature 1..21: note = synthesized primer
  source 1..21: mol_type = other DNA
aacccgccaggctctatgata

SEQ ID NO: 29 - DNA, 21 bp, synthetic construct
  misc_feature 1..21: note = synthesized primer
  source 1..21: mol_type = other DNA
caacatcgtcgtaatcggaca

SEQ ID NO: 30 - DNA, 21 bp, synthetic construct
  misc_feature 1..21: note = synthesized primer
  source 1..21: mol_type = other DNA
gtctaagacccaggcgtactt

SEQ ID NO: 31 - DNA, 20 bp, synthetic construct
  misc_feature 1..20: note = synthesized primer
  source 1..20: mol_type = other DNA
tgtcagtcatcgcccatgtg

SEQ ID NO: 32 - DNA, 21 bp, synthetic construct
  misc_feature 1..21: note = synthesized primer
  source 1..21: mol_type = other DNA
catccttgcgagtgtcagtga

SEQ ID NO: 33 - DNA, 21 bp, synthetic construct
  misc_feature 1..21: note = synthesized primer
  source 1..21: mol_type = other DNA
caagccagtacgcatcatgtg

SEQ ID NO: 34 - DNA, 22 bp, synthetic construct
  misc_feature 1..22: note = synthesized primer
  source 1..22: mol_type = other DNA
tgcttcctgtgtttcaaagtgt

SEQ ID NO: 35 - DNA, 21 bp, synthetic construct
  misc_feature 1..21: note = synthesized primer
  source 1..21: mol_type = other DNA
atgccctttgagctttgcttc

SEQ ID NO: 36 - DNA, 21 bp, synthetic construct
  misc_feature 1..21: note = synthesized primer
  source 1..21: mol_type = other DNA
aactggactggctgagagaac

SEQ ID NO: 37 - DNA, 19 bp, synthetic construct
  misc_feature 1..19: note = synthesized primer
  source 1..19: mol_type = other DNA
agccccatcactgtggagt

SEQ ID NO: 38 - DNA, 20 bp, synthetic construct
  misc_feature 1..20: note = synthesized primer
  source 1..20: mol_type = other DNA
gatgccgctcaacatcttgc

SEQ ID NO: 39 - DNA, 23 bp, synthetic construct
  misc_feature 1..23: note = synthesized primer
  source 1..23: mol_type = other DNA
tatcattgaccgctcctttaggt

SEQ ID NO: 40 - DNA, 19 bp, synthetic construct
  misc_feature 1..19: note = synthesized primer
  source 1..19: mol_type = other DNA
gctcgccttgatggttcct

SEQ ID NO: 41 - DNA, 23 bp, synthetic construct
  misc_feature 1..23: note = synthesized primer
  source 1..23: mol_type = other DNA
gcacatagagagaatgagcttcc

SEQ ID NO: 42 - DNA, 19 bp, synthetic construct
  misc_feature 1..19: note = synthesized primer
  source 1..19: mol_type = other DNA
ctccgctctgaacaaggct

SEQ ID NO: 43 - DNA, 21 bp, synthetic construct
  misc_feature 1..21: note = synthesized primer
  source 1..21: mol_type = other DNA
gcgtaccctgacaccaatctc

SEQ ID NO: 44 - DNA, 21 bp, synthetic construct
  misc_feature 1..21: note = synthesized primer
  source 1..21: mol_type = other DNA
ctcctcttcgcacttctgctc

SEQ ID NO: 45 - DNA, 21 bp, synthetic construct
  misc_feature 1..21: note = synthesized primer
  source 1..21: mol_type = other DNA
atgcccctcaacgtgaacttc

SEQ ID NO: 46 - DNA, 21 bp, synthetic construct
  misc_feature 1..21: note = synthesized primer
  source 1..21: mol_type = other DNA
cgcaacataggatggagagca

SEQ ID NO: 47 - DNA, 22 bp, synthetic construct
  misc_feature 1..22: note = synthesized primer
  source 1..22: mol_type = other DNA
ctccaagccaaagtccttagag

SEQ ID NO: 48 - DNA, 22 bp, synthetic construct
  misc_feature 1..22: note = synthesized primer
  source 1..22: mol_type = other DNA
aggagctgtcattagggacatc

SEQ ID NO: 49 - DNA, 23 bp, synthetic construct
  misc_feature 1..23: note = synthesized primer
  source 1..23: mol_type = other DNA
gttctcagcccaacaatacaaga

SEQ ID NO: 50 - DNA, 23 bp, synthetic construct
  misc_feature 1..23: note = synthesized primer
  source 1..23: mol_type = other DNA
gttctcagcccaacaatacaaga

SEQ ID NO: 51 - DNA, 21 bp, synthetic construct
  misc_feature 1..21: note = synthesized primer
  source 1..21: mol_type = other DNA
atggacgctgatggcaatacc

SEQ ID NO: 52 - DNA, 19 bp, synthetic construct
  misc_feature 1..19: note = synthesized primer
  source 1..19: mol_type = other DNA
tccccattcacgtctccca

SEQ ID NO: 53 - DNA, 19 bp, synthetic construct
  misc_feature 1..19: note = synthesized primer
  source 1..19: mol_type = other DNA
cccatccccaggagtcttg

SEQ ID NO: 54 - DNA, 21 bp, synthetic construct
  misc_feature 1..21: note = synthesized primer
  source 1..21: mol_type = other DNA
accatgactaggggcactgta

SEQ ID NO: 55 - DNA, 20 bp, synthetic construct
  misc_feature 1..20: note = synthesized primer
  source 1..20: mol_type = other DNA
ttcaccaccatggagaaggc

SEQ ID NO: 56 - DNA, 20 bp, synthetic construct
  misc_feature 1..20: note = synthesized primer
  source 1..20: mol_type = other DNA
ggcatggactgtggtcatga

SEQ ID NO: 57 - DNA, 21 bp, synthetic construct
  misc_feature 1..21: note = synthesized primer
  source 1..21: mol_type = other DNA
ggtgtgactacggagagaacc

SEQ ID NO: 58 - DNA, 20 bp, synthetic construct
  misc_feature 1..20: note = synthesized primer
  source 1..20: mol_type = other DNA
ggtagggtgggtgtcattcc

SEQ ID NO: 59 - DNA, 23 bp, synthetic construct
  misc_feature 1..23: note = synthesized primer
  source 1..23: mol_type = other DNA
atactccgatcaccaatgtacct

SEQ ID NO: 60 - DNA, 21 bp, synthetic construct
  misc_feature 1..21: note = synthesized primer
  source 1..21: mol_type = other DNA
gactgtctctgacactcctgt

SEQ ID NO: 61 - DNA, 21 bp, synthetic construct
  misc_feature 1..21: note = synthesized primer
  source 1..21: mol_type = other DNA
gccttgaccttatgtcatggg

SEQ ID NO: 62 - DNA, 19 bp, synthetic construct
  misc_feature 1..19: note = synthesized primer
  source 1..19: mol_type = other DNA
cctgtgctgtagtcgcact

SEQ ID NO: 63 - DNA, 23 bp, synthetic construct
  misc_feature 1..23: note = synthesized primer
  source 1..23: mol_type = other DNA
ggaagcaacacattggagaatgg

SEQ ID NO: 64 - DNA, 22 bp, synthetic construct
  misc_feature 1..22: note = synthesized primer
  source 1..22: mol_type = other DNA
ctttggtaggagtcacactgtc

SEQ ID NO: 65 - DNA, 22 bp, synthetic construct
  misc_feature 1..22: note = synthesized primer
  source 1..22: mol_type = other DNA
tgttggggtactcaagaactct

SEQ ID NO: 66 - DNA, 22 bp, synthetic construct
  misc_feature 1..22: note = synthesized primer
  source 1..22: mol_type = other DNA
ccctcccgtaataaggttcctg

SEQ ID NO: 67 - DNA, 21 bp, synthetic construct
  misc_feature 1..21: note = synthesized primer
  source 1..21: mol_type = other DNA
gaaaggaagccgcactcagtt

SEQ ID NO: 68 - DNA, 22 bp, synthetic construct
  misc_feature 1..22: note = synthesized primer
  source 1..22: mol_type = other DNA
cagacgtttgtagcaacagtca

SEQ ID NO: 69 - DNA, 19 bp, synthetic construct
  misc_feature 1..19: note = synthesized primer
  source 1..19: mol_type = other DNA
ctggcgctcagccatacag

SEQ ID NO: 70 - DNA, 23 bp, synthetic construct
  misc_feature 1..23: note = synthesized primer
  source 1..23: mol_type = other DNA
cgcacttatactggtcaaatccc

SEQ ID NO: 71 - DNA, 21 bp, synthetic construct
  misc_feature 1..21: note = synthesized primer
  source 1..21: mol_type = other DNA
tcctaacccttttgtcgcctg

SEQ ID NO: 72 - DNA, 19 bp, synthetic construct
  misc_feature 1..19: note = synthesized primer
  source 1..19: mol_type = other DNA
cgcttcccagaggatctgc

SEQ ID NO: 73 - DNA, 21 bp, synthetic construct
  misc_feature 1..21: note = synthesized primer
  source 1..21: mol_type = other DNA
tgtgggcatcaatggatttgg

SEQ ID NO: 74 - DNA, 22 bp, synthetic construct
  misc_feature 1..22: note = synthesized primer
  source 1..22: mol_type = other DNA
acaccatgtattccgggtcaat